European Patent Specification EP 3 598 899 B1, published November 15, 2023. Title: PLANT GROWTH-PROMOTING MICROBES AND USES THEREFOR. Applicant: MONSANTO TECHNOLOGY LLC. The sequence listing filed with the application follows.

SEQUENCE LISTING (11 sequences)

SEQ ID NO: 1 - DNA, 1436 bp, Pantoea agglomerans
  misc_feature: SGI bacterial isolate SGI-003_H11
  misc_feature: encodes a 16S ribosomal RNA
  misc_feature (62)..(63): n is a, c, g, or t
gctggcggcaggcctaacacatgcaagtcgagcggtagcacagagagcttgctctcgggtgnngagcggcggacgggtgagtaatgtctgggaaactgcctgatggagggggataactactggaaacggtagctaataccgcataacgtcgcaagaccaaagtgggggaccttcgggcctcatgccatcagatgtgcccagatgggattagctagtaggtgaggtaatggctcacctaggcgacgatccctagctggtctgagaggatgaccagccacactggaactgagacacggtccagactcctacgggaggcagcagtggggaatattgcacaatgggcgcaagcctgatgcagccatgccgcgtgtatgaagaaggccttcgggttgtaaagtactttcagcgaggaggaaggcgataaggttaataaccttgtcgattgacgttactcgcagaagaagcaccggctaactccgtgccagcagccgcggtaatacggagggtgcaagcgttaatcggaattactgggcgtaaagcgcacgcaggcggtctgtcaagtcggatgtgaaatccccgggctcaacctgggaactgcatccgaaactggcaggctagagtcttgtagaggggggtagaattccaggtgtagcggtgaaatgcgtagagatctggaggaataccggtggcgaaggcggccccctggacaaagactgacgctcaggtgcgaaagcgtggggagcaaacaggattagataccctggtagtccacgctgtaaacgatgtcgacttggaggttgttcccttgaggagtggcttccggagctaacgcgttaagtcgaccgcctggggagtacggccgcaaggttaaaactcaaatgaattgacgggggcccgcacaagcggtggagcatgtggtttaattcgatgcaacgcgaagaaccttacctactcttgacatccagagaacttagcagagatgctttggtgccttcgggaactctgagacaggtgctgcatggctgtcgtcagctcgtgttgtgaaatgttgggttaagtcccgcaacgagcgcaacccttatcctttgttgccagcggttcggccgggaactcaaaggagactgccagtgataaactggaggaaggtggggatgacgtcaagtcatcatggcccttacgagtagggctacacacgtgctacaatggcatatacaaagagaagcgacctcgcgagagcaagcggacctcataaagtatgtcgtagtccggatcggagtctgcaactcgactccgtgaagtcggaatcgctagtaatcgtggatcagaatgccacggtgaatacgttcccgggccttgtacacaccgcccgtcacaccatgggagtgggttgcaaaagaagtaggtagcttaaccttcgggagggcgcttaccacttt

SEQ ID NO: 2 - DNA, 1440 bp, Bacillus thuringiensis
  misc_feature: SGI bacterial isolate SGI-020_A01
  misc_feature: encodes a 16S ribosomal RNA
cgtgcctaatacatgcaagtcgagcgaatggattaagagcttgctcttatgaagttagcggcggacgggtgagtaacacgtgggtaacctgcccataagactgggataactccgggaaaccggggctaataccggataatattttgaactgcatggttcgaaattgaaaggcggcttcggctgtcacttatggatggacccgcgtcgcattagctagttggtgaggtaacggctcaccaaggcaacgatgcgtagccgacctgagagggtgatcggccacactgggactgagacacggcccagactcctacgggaggcagcagtagggaatcttccgcaatggacgaaagtctgacggagcaacgccgcgtgagtgatgaaggctttcgggtcgtaaaactctgttgttagggaagaacaagtgctagttgaataagctggcaccttgacggtacctaaccagaaagccacggctaactacgtgccagcagccgcggtaatacgtaggtggcaagcgttatccggaattattgggcgtaaagcgcgcgcaggtggtttcttaagtctgatgtgaaagcccacggctcaaccgtggagggtcattggaaactgggagacttgagtgcagaagaggaaagtggaattccatgtgtagcggtgaaatgcgtagagatatggaggaacaccagtggcgaaggcgactttctggtctgtaactgacactgaggcgcgaaagcgtggggagcaaacaggattagataccctggtagtccacgccgtaaacgatgagtgctaagtgttagagggtttccgccctttagtgctgaagttaacgcattaagcactccgcctggggagtacggccgcaaggctgaaactcaaaggaattgacgggggcccgcacaagcggtggagcatgtggtttaattcgaagcaacgcgaagaaccttaccaggtcttgacatcctctgaaaaccctagagatagggcttctccttcgggagcagagtgacaggtggtgcatggttgtcgtcagctcgtgtcgtgagatgttgggttaagtcccgcaacgagcgcaacccttgatcttagttgccatcattaagttgggcactctaaggtgactgccggtgacaaaccggaggaaggtggggatgacgtcaaatcatcatgccccttatgacctgggctacacacgtgctacaatggacggtacaaagagctgcaagaccgcgaggtggagctaatctcataaaaccgttctcagttcggattgtaggctgcaactcgcctacatgaagctggaatcgctagtaatcgcggatcagcatgccgcggtgaatacgttcccgggccttgtacacaccgcccgtcacaccacgagagtttgtaacacccgaagtcggtggggtaacctttttggagccagccgcctaaggt

SEQ ID NO: 3 - DNA, 1414 bp, Burkholderia metallica
  misc_feature: SGI bacterial isolate SGI-026_G06
  misc_feature: encodes a 16S ribosomal RNA
catgcaagtcgaacggcagcacgggtgcttgcacctggtggcgagtggcgaacgggtgagtaatacatcggaacatgtcctgtagtgggggatagcccggcgaaagccggattaataccgcatacgatctacggatgaaagcgggggaccttcgggcctcgcgctatagggttggccgatggctgattagctagttggtggggtaaaggcctaccaaggcgacgatcagtagctggtctgagaggacgaccagccacactgggactgagacacggcccagactcctacgggaggcagcagtggggaattttggacaatgggcgaaagcctgatccagcaatgccgcgtgtgtgaagaaggccttcgggttgtaaagcacttttgtccggaaagaaatccttgattctaatacagtcgggggatgacggtaccggaagaataagcaccggctaactacgtgccagcagccgcggtaatacgtagggtgcgagcgttaatcggaattactgggcgtaaagcgtgcgcaggcggtttgctaagaccgatgtgaaatccccgggctcaacctgggaactgcattggtgactggcaggctagagtatggcagaggggggtagaattccacgtgtagcagtgaaatgcgtagagatgtggaggaataccgatggcgaaggcagccccctgggccaatactgacgctcatgcacgaaagcgtggggagcaaacaggattagataccctggtagtccacgccctaaacgatgtcaactagttgttggggattcatttccttagtaacgtagctaacgcgtgaagttgaccgcctggggagtacggtcgcaagattaaaactcaaaggaattgacggggacccgcacaagcggtggatgatgtggattaattcgatgcaacgcgaaaaaccttacctacccttgacatggtcggaatcctgctgagaggcgggagtgctcgaaagagaaccggcgcacaggtgctgcatggctgtcgtcagctcgtgtcgtgagatgttgggttaagtcccgcaacgagcgcaacccttgtccttagttgctacgcaagagcactctaaggagactgccggtgacaaaccggaggaaggtggggatgacgtcaagtcctcatggcccttatgggtagggcttcacacgtcatacaatggtcggaacagagggttgccaacccgcgagggggagctaatcccagaaaaccgatcgtagtccggattgcactctgcaactcgagtgcatgaagctggaatcgctagtaatcgcggatcagcatgccgcggtgaatacgttcccgggtcttgtacacaccgcccgtcacaccatgggagtgggttttaccagaagtggctagtctaaccgcaaggaggacggtcaccacggtagga

SEQ ID NO: 4 - DNA, 1423 bp, Burkholderia vietnamiensis
  misc_feature: SGI bacterial isolate SGI-026_G07
  misc_feature: encodes a 16S ribosomal RNA
tgccttacacatgcaagtcgaacggcagcacgggtgcttgcacctggtggcgagtggcgaacgggtgagtaatacatcggaacatgtcctgtagtgggggatagcccggcgaaagccggattaataccgcatacgatctaaggatgaaagcgggggaccttcgggcctcgcgctatagggttggccgatggctgattagctagttggtggggtaaaggcctaccaaggcgacgatcagtagctggtctgagaggacgaccagccacactgggactgagacacggcccagactcctacgggaggcagcagtggggaattttggacaatgggcgaaagcctgatccagcaatgccgcgtgtgtgaagaaggccttcgggttgtaaagcacttttgtccggaaagaaatccttggctctaatacagtcgggggatgacggtaccggaagaataagcaccggctaactacgtgccagcagccgcggtaatacgtagggtgcaagcgttaatcggaattactgggcgtaaagcgtgcgcaggcggtttgctaagaccgatgtgaaatccccgggctcaacctgggaactgcattggtgactggcaggctagagtatggcagaggggggtagaattccacgtgtagcagtgaaatgcgtagagatgtggaggaataccgatggcgaaggcagccccctgggccaatactgacgctcatgcacgaaagcgtggggagcaaacaggattagataccctggtagtccacgccctaaacgatgtcaactagttgttggggattcatttccttagtaacgtagctaacgcgtgaagttgaccgcctggggagtacggtcgcaagattaaaactcaaaggaattgacggggacccgcacaagcggtggatgatgtggattaattcgatgcaacgcgaaaaaccttacctacccttgacatggtcggaagcccgatgagagttgggcgtgctcgaaagagaaccggcgcacaggtgctgcatggctgtcgtcagctcgtgtcgtgagatgttgggttaagtcccgcaacgagcgcaacccttgtccttagttgctacgcaagagcactctaaggagactgccggtgacaaaccggaggaaggtggggatgacgtcaagtcctcatggcccttatgggtagggcttcacacgtcatacaatggtcggaacagagggttgccaacccgcgagggggagctaatcccagaaaaccgatcgtagtccggattgcactctgcaactcgagtgcatgaagctggaatcgctagtaatcgcggatcagcatgccgcggtgaatacgttcccgggtcttgtacacaccgcccgtcacaccatgggagtgggttttaccagaagtggctagtctaaccgcaaggaggacggtcaccacggtagga

SEQ ID NO: 5 - DNA, 1441 bp, Bacillus pumilus
  misc_feature: SGI bacterial isolate SGI-034_C09
  misc_feature: encodes a 16S ribosomal RNA
  misc_feature (605)..(605): n is a, c, g, or t
gcggcgtgcctaatacatgcaagtcgagcggacagaagggagcttgctcccggatgttagcggcggacgggtgagtaacacgtgggtaacctgcctgtaagactgggataactccgggaaaccggagctaataccggatagttccttgaaccgcatggttcaaggatgaaagacggtttcggctgtcacttacagatggacccgcggcgcattagctagttggtgaggtaacggctcaccaaggcgacgatgcgtagccgacctgagagggtgatcggccacactgggactgagacacggcccagactcctacgggaggcagcagtagggaatcttccgcaatggacgaaagtctgacggagcaacgccgcgtgagtgatgaaggttttcggatcgtaaagctctgttgttagggaagaacaagtgcaagagtaactgcttgcaccttgacggtacctaaccagaaagccacggctaactacgtgccagcagccgcggtaatacgtaggtggcaagcgttgtccggaattattgggcgtaaagggctcgcaggcggtttcttaagtctgatgtgaaagcccccggctcaaccggggagggtcatnggaaactgggaaacttgagtgcagaagaggagagtggaattccacgtgtagcggtgaaatgcgtagagatgtggaggaacaccagtggcgaaggcgactctctggtctgtaactgacgctgaggagcgaaagcgtggggagcgaacaggattagataccctggtagtccacgccgtaaacgatgagtgctaagtgttagggggtttccgccccttagtgctgcagctaacgcattaagcactccgcctggggagtacggtcgcaagactgaaactcaaaggaattgacgggggcccgcacaagcggtggagcatgtggtttaattcgaagcaacgcgaagaaccttaccaggtcttgacatcctctgacaaccctagagatagggctttcccttcggggacagagtgacaggtggtgcatggttgtcgtcagctcgtgtcgtgagatgttgggttaagtcccgcaacgagcgcaacccttgatcttagttgccagcattcagttgggcactctaaggtgactgccggtgacaaaccggaggaaggtggggatgacgtcaaatcatcatgccccttatgacctgggctacacacgtgctacaatggacagaacaaagggctgcgagaccgcaaggtttagccaatcccacaaatctgttctcagttcggatcgcagtctgcaactcgactgcgtgaagctggaatcgctagtaatcgcggatcagcatgccgcggtgaatacgttcccgggccttgtacacaccgcccgtcacaccacgagagtttgcaacacccgaagtcggtgaggtaacctttatggagccagccgccgaaggt

SEQ ID NO: 6 - DNA, 1410 bp, Herbaspirillum sp.
  misc_feature: SGI bacterial isolate SGI-034_E10
  misc_feature: encodes a 16S ribosomal RNA
tgcaagtcgaaacggcagcataggagcttgctcctgatggcgagtggcgaacgggtgagtaatatatcggaacgtgccctagagtgggggataactagtcgaaagactagctaataccgcatacgatctacggatgaaagtgggggatcgcaagacctcatgctcctggagcggccgatatctgattagctagttggtggggtaaaagcctaccaaggcaacgatcagtagctggtctgagaggacgaccagccacactgggactgagacacggcccagactcctacgggaggcagcagtggggaattttggacaatgggggcaaccctgatccagcaatgccgcgtgagtgaagaaggccttcgggttgtaaagctcttttgtcagggaagaaacggtagtagcgaataactattactaatgacggtacctgaagaataagcaccggctaactacgtgccagcagccgcggtaatacgtagggtgcaagcgttaatcggaattactgggcgtaaagcgtgcgcaggcggttgtgtaagtcagatgtgaaatccccgggctcaacctgggaattgcatttgagactgcacggctagagtgtgtcagaggggggtagaattccacgtgtagcagtgaaatgcgtagatatgtggaggaataccgatggcgaaaggcagccccctgggataacactgacgctcatgcacgaaagcgtggggagcaaacaggattagataccctggtagtccacgccctaaacgatgtctactagttgtcgggtcttaattgacttggtaacgcagctaacgcgtgaagtagaccgcctggggagtacggtcgcaagattaaaactcaaaggaattgacggggacccgcacaagcggtggatgatgtggattaattcgatgcaacgcgaaaaaccttacctacccttgacatggatggaatcctgaagagatttgggagtgctcgaaagagaaccatcacacaggtgctgcatggctgtcgtcagctcgtgtcgtgagatgttgggttaagtcccgcaacgagcgcaacccttgtcattagttgctacgaaagggcactctaatgagactgccggtgacaaaccggaggaaggtggggatgacgtcaagtcctcatggcccttatgggtagggcttcacacgtcatacaatggtacatacagagggccgccaacccgcgagggggagctaatcccagaaagtgtatcgtagtccggattggagtctgcaactcgactccatgaagttggaatcgctagtaatcgcggatcagcatgtcgcggtgaatacgttcccgggtcttgtacacaccgcccgtcacaccatgggagcgggttttaccagaagtgggtagcctaaccgcaaggagggcgctcaccacggt

SEQ ID NO: 7 - DNA, 1368 bp, Pedobacter sp.
  misc_feature: SGI bacterial isolate SGI-041_B03
  misc_feature: encodes a 16S ribosomal RNA
  misc_feature (529)..(529): n is a, c, g, or t
gaaagtggcgcacgggtgcgtaacgcgtatgcaacctaccttcatctgggggatagcccggagaaatccggattaataccgcataaaatcacagtactgcatagtgcaatgatcaaacatttatgggaagaagatgggcatgcgtgtcattagctagttggcggggtaacggcccaccaaggcgacgatgactaggggatctgagaggatggccccccacactggtactgagacacggaccagactcctacgggaggcagcagtaaggaatattggtcaatggaggcaactctgaaccagccatgccgcgtgcaggaagactgccctatgggttgtaaactgcttttatccgggaataaacctgagtacgtgtacttagctgaatgtaccggaagaataaggatcggctaactccgtgccagcagccgcggtaatacggaggatccaagcgttatccggatttattgggtttaaagggtgcgtaggcggcctgttaagtcaggggtgaaagacggtagctcaactatcngcagtgcccttgatactgatgggcttgaatggactagaggtaggcggaatgagacaagtagcggtgaaatgcatagatatgtctcagaacaccgattgcgaaggcagcttactatggtcttattgacgctgaggcacgaaagcgtggggatcaaacaggattagataccctggtagtccacgccctaaacgatgaacactcgctgttggcgatacacagtcagcggctaagcgaaagcgttaagtgttccacctggggagtacgctcgcaagagtgaaactcaaaggaattgacgggggcccgcacaagcggaggagcatgtggtttaattcgatgatacgcgaggaaccttacccgggcttgaaagttagtgaatcatttagagataaatgagtgagcaatcacacgaaactaggtgctgcatggctgtcgtcagctcgtgccgtgaggtgttgggttaagtcccgcaacgagcgcaacccctatgtttagttgccagcacgttatggtggggactctaaacagactgcctgtgcaaacagagaggaaggaggggacgacgtcaagtcatcatggcccttacgtccggggctacacacgtgctacaatggatggtacagagggcagctacatagcaatatgatgcgaatctcacaaagccattcacagttcggattggggtctgcaactcgaccccatgaagttggattcgctagtaatcgcgtatcagcaatgacgcggtgaatacgttcccgggccttgtacacaccgcccgtcaagccatggaagttgggggtacctaaagtatgtaaccgcaaggagcgtcctagggtaaaacc

SEQ ID NO: 8 - DNA, 39 bp, Artificial sequence
  PCR primer M13-27F
tgtaaaacgacggccagttagagtttgatcctggctcag

SEQ ID NO: 9 - DNA, 37 bp, Artificial sequence
  PCR primer 1492R M13-tailed
caggaaacagctatgaccggttaccttgttacgactt

SEQ ID NO: 10 - DNA, 1059 bp, Pantoea agglomerans
atggctatcgacgaaaacaaacagaaagcgttggcggcagcactgggccagatcgaaaaacagttcggtaaaggctccatcatgcgcctgggtgaagaccgttccatggacgtggaaactatctccaccggttcgctttccctggatatcgccctcggcgctggcggtctgccaatgggccgtatcgtcgaaatctacgggcctgaatcttccggtaaaacgacgctgaccctgcaggttatcgccgccgcgcagcgtgaaggtaaaacctgtgcctttatcgatgcagagcacgcgctggatccggtatatgcccgcaagctgggcgtcgatatcgacaacctgctgtgctctcagccggacaccggcgaacaggcgcttgagatctgtgacgcgctggcgcgctccggtgcggtagacgtgctggtggtcgactccgttgcggcgctgacgccgaaagcggaaatcgaaggcgagatcggcgactctcacatgggcctcgcggcgcgtatgatgagccaggcaatgcgtaagctggccggtaacctgaagcagtccaacacgctgctgatcttcatcaaccagatccgtatgaaaattggcgtgatgttcggtaacccggaaaccaccaccggcggtaacgcgctgaaattctacgcctccgtgcgtctggatatccgccgtatcggtgcggtaaaagatggcgataacgtcattggtagcgaaacccgcgtgaaggtcgtgaagaacaaaatcgccgcgccgttcaagcaggcggagttccagatcctctacggcgaaggcatcaacttcttcggcgagctggtcgatctgggcgtgaaagagaagctgattgaaaaagcgggcgcctggtatagctacaacggcgacaaaattggtcagggtaaagcgaacgctatctcctggctgaaagagaacccggctgcggcgaaagagatcgagaagaaagttcgtgaactgctgctgaacaaccaggatgccacgccggacttcgcggttgatggtaaaagcgaagaagcaagcgaacaggatttctga

SEQ ID NO: 11 - protein, 352 aa, Pantoea agglomerans
MAIDENKQKALAAALGQIEKQFGKGSIMRLGEDRSMDVETISTGSLSLDIALGAGGLPMGRIVEIYGPESSGKTTLTLQVIAAAQREGKTCAFIDAEHALDPVYARKLGVDIDNLLCSQPDTGEQALEICDALARSGAVDVLVVDSVAALTPKAEIEGEIGDSHMGLAARMMSQAMRKLAGNLKQSNTLLIFINQIRMKIGVMFGNPETTTGGNALKFYASVRLDIRRIGAVKDGDNVIGSETRVKVVKNKIAAPFKQAEFQILYGEGINFFGELVDLGVKEKLIEKAGAWYSYNGDKIGQGKANAISWLKENPAAAKEIEKKVRELLLNNQDATPDFAVDGKSEEASEQDF